European Patent Specification EP 4 010 705 B1, published July 9, 2025. Title: Method of identifying peptide antigens and uses thereof. Applicant: HUMANITAS MIRASOLE S.P.A.; HUMANITAS UNIVERSITY. The sequence listing filed with the application follows.

SEQUENCE LISTING (80 sequences)

SEQ ID NO: 1 - protein, 15 aa, Homo sapiens
LGLALNFSVFYYEIL

SEQ ID NO: 2 - protein, 14 aa, Homo sapiens
LGLALNFSVFYYEI

SEQ ID NO: 3 - protein, 14 aa, Homo sapiens
LGLALNYSVFYYEI

SEQ ID NO: 4 - protein, 14 aa, Homo sapiens
LGLALNFSVFHYEI

SEQ ID NO: 5 - protein, 25 aa, Homo sapiens
EPVQLETLSIRGNNIRYFILPDSLP

SEQ ID NO: 6 - protein, 15 aa, Homo sapiens
LTTNLINLLAENGRL

SEQ ID NO: 7 - protein, 13 aa, Homo sapiens
LTANLIHLSENRL

SEQ ID NO: 8 - protein, 7 aa, Canis lupus familiaris
LGLALNF

SEQ ID NO: 9 - protein, 14 aa, Canis lupus familiaris
TSNLINLLAENGRL

SEQ ID NO: 10 - protein, 8 aa, Canis lupus familiaris
LMNLLANG

SEQ ID NO: 11 - protein, 9 aa, Felis catus
LGNFSVFYY

SEQ ID NO: 12 - protein, 7 aa, Felis catus
LNFGVFY

SEQ ID NO: 13 - protein, 15 aa, Felis catus
LTCNLINLLAENGRL

SEQ ID NO: 14 - protein, 15 aa, Mus musculus
LTANLMNLLAENGRL

SEQ ID NO: 15 - protein, 22 aa, Mus musculus
SAPLSQQWTAGMGLLLALIVLL

SEQ ID NO: 16 - protein, 18 aa, Mus musculus
KALKTLGIIMGVFTLCWL

SEQ ID NO: 17 - protein, 16 aa, Mus musculus
HRDLVPDRLFVFFNWL

SEQ ID NO: 18 - protein, 255 aa, Homo sapiens
MDDREDLVYQAKLAEQAERYDEMVESMKKVAGMDVELTVEERNLLSVAYKNVIGARRASWRIISSIEQKEENKGGEDKLKMIREYRQMVETELKLICCDILDVLDKHLIPAANTGESKVFYYKMKGDYHRYLAEFATGNDRKEAAENSLVAYKAASDIAMTELPPTHPIRLGLALNFSVFYYEILNSPDRACRLAKAAFDDAIAELDTLSEESYKDSTLIMQLLRDNLTLWTSDMQGDGEEQNKEALQDVEDENQ

SEQ ID NO: 19 - protein, 240 aa, Homo sapiens
MDDREDLVYQAKLAEQAERYDEMVESMKKVAGMDVELTVEERNLLSVAYKNVIGARRASWRIISSIEQKEENKGGEDKLKMIREYRQMVETELKLICCDILDVLDKHLIPAANTGESKVFYYKMKGDYHRYLAEFATGNDRKEAAENSLVAYKAASDIAMTELPPTHPIRLGLALNFSVFYYEILNSPDRACRLAKAAFDDAIAELDTLSEESYKDSTLIMQLLRDNLTLWTSDMQGDDS

SEQ ID NO: 20 - protein, 218 aa, Homo sapiens
MVESMKKVAGMDVELTVEERNLLSVAYKNVIGARRASWRIISSIEQKEENKGGEDKLKMIREYRQMVETELKLICCDILDVLDKHLIPAANTGESKVFYYKMKGDYHRYLAEFATGNDRKEAAENSLVAYKAASDIAMTELPPTHPIRLGLALNFSVFYYEILNSPDRACRLAKAAFDDAIAELDTLSEESYKDSTLIMQLLRDNLTLWTSDMQGDDS

SEQ ID NO: 21 - protein, 244 aa, Homo sapiens
MTMDKSELVQKAKLAEQAERYDDMAAAMKAVTEQGHELSNEERNLLSVAYKNVVGARRSSWRVISSIEQKTERNEKKQQMGKEYREKIEAELQDICNDVLELLDKYLIPNATQPESKVFYLKMKGDYFRYLSEVASGDNKQTTVSNSQQAYQEAFEISKKEMQPTHPIRLGLALNFSVFYYEILNSPEKACSLAKTAFDEAIAELDTLNEESYKDSTLIMQLLRDNLTLWTSENQGDEGDAGEG

SEQ ID NO: 22 - protein, 245 aa, Homo sapiens
MEKTELIQKAKLAEQAERYDDMATCMKAVTEQGAELSNEERNLLSVAYKNVVGGRRSAWRVISSIEQKTDTSDKKLQLIKDYREKVESELRSICTTVLELLDKYLIANATNPESKVFYLKMKGDYFRYLAEVACGDDRKQTIDNSQGAYQEAFDISKKEMQPTHPIRLGLALNFSVFYYEILNNPELACTLAKTAFDEAIAELDTLNEDSYKDSTLIMQLLRDNLTLWTSDSAGEECDAAEGAEN

SEQ ID NO: 23 - protein, 253 aa, Homo sapiens
MDKNELVQKAKLAEQAERYDDMAACMKSVTEQGAELSNEERNLLSVAYKNVVGARRSSWRVVSSIEQKTEGAEKKQQMAREYREKIETELRDICNDVLSLLEKFLIPNASQAESKVFYLKMKGDYYRYLAEVAAGDDKKGIVDQSQQAYQEAFEISKKEMQPTHPIRLGLALNFSVFYYEILNSPEKACSLAKTAFDEAIAELDTLSEESYKDSTLIMQLLRDNLTLWTSDTQGDEAEAGEGGENSDMQGDDS

SEQ ID NO: 24 - protein, 246 aa, Homo sapiens
MGDREQLLQRARLAEQAERYDDMASAMKAVTELNEPLSNEDRNLLSVAYKNVVGARRSSWRVISSIEQKTMADGNEKKLEKVKAYREKIEKELETVCNDVLSLLDKFLIKNCNDFQYESKVFYLKMKGDYYRYLAEVASGEKKNSVVEASEAAYKEAFEISKEQMQPTHPIRLGLALNFSVFYYEIQNAPEQACLLAKQAFDDAIAELDTLNEDSYKDSTLIMQLLRDNLTLWTSDQQDEEAGEGN

SEQ ID NO: 25 - protein, 247 aa, Homo sapiens
MVDREQLVQKARLAEQAERYDDMAAAMKNVTELNEPLSNEERNLLSVAYKNVVGARRSSWRVISSIEQKTSADGNEKKIEMVRAYREKIEKELEAVCQDVLSLLDNYLIKNCSETQYESKVFYLKMKGDYYRYLAEVATGEKRATVVESSEKAYSEAHEISKEHMQPTHPIRLGLALNYSVFYYEIQNAPEQACHLAKTAFDDAIAELDTLNEDSYKDSTLIMQLLRDNLTLWTSDQQDDDGGEGNN

SEQ ID NO: 26 - protein, 248 aa, Homo sapiens [sequence omitted]

SEQ ID NO: 27 - protein, 119 aa, Homo sapiens
MKLVRFLMKLSHETVTIELKNGTQVHGTITGVDVSMNTHLKAVKMTLKNREPVQLETLSIRGNNIRYFILPDSLPLDTLLVDVEPKVKSKKREAVAGRGRGRGRGRGRGRGRGRGGPRR

SEQ ID NO: 28 - protein, 213 aa, Homo sapiens
MAAPAVSGLSRQVRCFSTSVVRPFAKLVRPPVQVYGIEGRYATALYSAASKQNKLEQVEKELLRVAQILKEPKVAASVLNPYVKRSIKVKSLNDITAKERFSPLTTNLINLLAENGRLSNTQGVVSAFSTMMSVHRGEVPCTVTSASPLEEATLSELKTVLKSFLSQGQVLKLEAKTDPSILGGMIVRIGEKYVDMSVKTKIQKLGRAMREIV

SEQ ID NO: 29 - protein, 858 aa, Homo sapiens [sequence omitted]

SEQ ID NO: 30 - protein, 262 aa, Canis lupus familiaris
MDDREDLVYQAKLAEQAERYDVQMAFCDEMVESMKKVAGMDVELTVEERNLLSVAYKNVIGARRASWRIISSIEQKEENKGGEDKLKMIREYRQMVETELKLICCDILDVLDKHLIPAANTGESKVFYYKMKGDYHRYLAEFATGNDRKEAAENSLVAYKAASDIAMTELPPTHPIRLGLALNFSVFYYEILNSPDRACRLAKAAFDDAIAELDTLSEESYKDSTLIMQLLRDNLTLWTSDMQGDGEEQNKEALQDVEDENQ

SEQ ID NO: 31 - protein, 255 aa, Canis lupus familiaris; identical to SEQ ID NO: 18

SEQ ID NO: 32 - protein, 224 aa, Canis lupus familiaris
MAFCDEMVESMKKVAGMDVELTVEERNLLSVAYKNVIGARRASWRIISSIEQKEENKGGEDKLKMIREYRQMVETELKLICCDILDVLDKHLIPAANTGESKVFYYKMKGDYHRYLAEFATGNDRKEAAENSLVAYKAASDIAMTELPPTHPIRLGLALNFSVFYYEILNSPDRACRLAKAAFDDAIAELDTLSEESYKDSTLIMQLLRDNLTLWTSDMQGDDS

SEQ ID NO: 33 - protein, 267 aa, Canis lupus familiaris
MIKYLFAEAGKILQDVFSLPSCCSLLVQMAFCDEMVESMKKVAGMDVELTVEERNLLSVAYKNVIGARRASWRIISSIEQKEENKGGEDKLKMIREYRQMVETELKLICCDILDVLDKHLIPAANTGESKVFYYKMKGDYHRYLAEFATGNDRKEAAENSLVAYKAASDIAMTELPPTHPIRLGLALNFSVFYYEILNSPDRACRLAKAAFDDAIAELDTLSEESYKDSTLIMQLLRDNLTLWTSDMQGDGEEQNKEALQDVEDENQ

SEQ ID NO: 34 - protein, 247 aa, Canis lupus familiaris
MEKTELIQKAKLAEQAEQAERYDDRATCVMAGPEQGAELSNEERSLLSVAYKNVVGGRRSAWRVSSSIEQKTDTSDKKLQLIKDCREKVESELRSICTTTLELLDKYLTANATNPESKVFYLKMKGDYFRYLAEVARGDDRKQTIDNSQGAYQEAFDISKKEMQPTHPIRLGLALNFSVFYYEILNNPELVCTLAKTAFDEAIAELGTLNEDSYKDSTLIMQLLRDNLTRTSDSAGEECDAAEGAEN

SEQ ID NO: 35 - protein, 245 aa, Canis lupus familiaris; identical to SEQ ID NO: 22

SEQ ID NO: 36 - protein, 245 aa, Canis lupus familiaris
MDKNELVQKAKLAEQAERYDDMAACMKSVTEQGAELSNEERNLLSVAYKNVVGARRSSWRVVSSIEQKTEGAEKKQQMAREYREKIETELRDICNDVLSLLEKFLIPNASQAESKVFYLKMKGDYYRYLAEVAAGDDKKGIVDQSQQAYQEAFEISKKEMQPTHPIRLGLALNFSVFYYEILNSPEKACSLAKTAFDEAIAELDTLSEESYKDSTLIMQLLRDNLTLWTSDTQGDEAEAGEGGEN

SEQ ID NO: 37 - protein, 244 aa, Canis lupus familiaris
MDKSELVQKAKLAEQAERYDDMAAAMKAVTEQGHELSNEERNLLSVAYKNVVGARRSSWRVISSIEQKTERNEKKQQMGKEYREKIEAELQDICNDVLELLDKYLIPNATQPESKVFYLKMKGDYFRYLSEVASGDNKQTTVSNSQQAYQEAFEISKKEMQPTHPIRLGLALNFSVFYYEILNSPEKACSLAKTAFDEAIAELDTLNEESYKDSTLIMQLLRDNLTLWTSENQGDEGDAGEGEN

SEQ ID NO: 38 - protein, 246 aa, Canis lupus familiaris
MGDREQLLQRARLAEQAERYDDMASAMKAVTELNEPLSNEDRNLLSVAYKNVVGARRSSWRVISSIEQKTMADGNEKKLEKVKAYREKIEKELETVCNDVLALLDKFLIKNCNDFQYESKVFYLKMKGDYYRYLAEVASGEKKNSVVEASEAAYKEAFEISKEHMQPTHPIRLGLALNFSVFYYEIQNAPEQACLLAKQAFDDAIAELDTLNEDSYKDSTLIMQLLRDNLTLWTSDQQDEEAGEGN

SEQ ID NO: 39 - protein, 232 aa, Canis lupus familiaris
MSFCLISSSQPENKVTELNEPLSNEERNLLSVAYKNVVGARRSSWRVISSIEQKTSADGNEKKIEMVRAYREKIEKELEAVCQDVLSLLDNYLIKNCSETQYESKVFYLKMKGDYYRYLAEVATGEKRATVVESSEKAYSEAHEISKEHMQPTHPIRLGLALNYSVFYYEIQNAPEQACHLAKTAFDDAIAELDTLNEDSYKDSTLIMQLLRDNLTLWTSDQQDDDGGEGNN

SEQ ID NO: 40 - protein, 248 aa, Canis lupus familiaris
MERASLIQKAKLAEQAERYEDMAAFMKSAVEKGEELSCEERNLLSVAYKNVVGGQRAAWRVLSSIEQKGNEESSEEKGPEVREYREKVETELRGVCDTVLGLLDSHLIKEAGDAESRVFYLKMKGDYYRYLAEVATGDDKKRIIDSARSAYQEAMDISKKEMPPTNPIRLGLALNFSVFHYEIANSPEEAISLAKTTFDEAMADLHTLSEDSYKDSTLIMQLLRDNLTLWTADNAGEEGGEAPEEPQS

SEQ ID NO: 41 - protein, 507 aa, Canis lupus familiaris
MGAGGPRRGEGPPDGGWGWAVLGACFVVTGFAYGFPKAVSVFFRALMRDFGAGYSDTAWVSSIMLAMLYGTGPVSSILVTRFGCRPVMLVGGLLASAGMVLASFATRLLELYLTAGVLTGLGLALNFQPSLIMLGLYFERRRPLANGLAAAGSPVFLSTLSPLGQQLLEHFGWRGGFLLLGGLLLHCCACGAVMRPPPGPGPRPRRDSADDPPADADAEAGAGADAERPGLRLREAPPGGRPRRRLLDVAVCADRAFAVYTVTNFLMALGLFVPAILLVWAKDAGVPDADAAFLLSVVGFVDIVARPACGALAGLARLRPHVAYLFSLALVANGLTDLSSARARSYGALVAFCVAFGLSYGMVGALQFEVLMAAVGSLRFPSALGLVLLVEAVAVLIGPPSAGRLVDALKNYEIIFYLAGSEVALAGIFMAVATKCCLRRSRDTPPGQVAEGGASDTEDAEAEVDSEALPTGAEEPGSREPLEVPSPGARPAEAEVEAGPGRDTKSV

SEQ ID NO: 42 - protein, 498 aa, Canis lupus familiaris
MPPAVGGPVGYTPPDGGWGWAVVVGAFISIGFSYAFPKSITVFFKEIESIFSATTSEVSWISSIMLAVMYGGGPISSILVNKYGSRPIMIVGGCLSGCGLIAASFCNTVQELYLCIGVIGGLGLAFNLNPALTMIGKYFYKRRPLANGLAMAGSPVFLSTLAPLNQAFFGIFGWRGSFLILGGLLLNCCVAGALMRPIGPPPTSAGKDRSKESLQEAEKSDEKKGGDANTDLIGGNRKEEKGSVFQTINKFLDLSLFTHRGFLLYLSGNVLMFFGLFTPLVFLSNYGKSQHYSSEKSAFLLSILAFVDMVARPSMGLVANTKWIRPRVQYFFAASIVANGVCHLLAPLSSSYIGFCVYAGFFGFAFGWLSSVLFETLMDLVGPQRFSSAVGLVTIVECCPVLLGPPLLGRLNDIYGDYKYTYWACGVILIIAGIYLFIGMGINYQLVAKEQKAEKQQKKESKEEETSVDAAEKPKEYASESAEQKDTEGSPKEEESPV

SEQ ID NO: 43 - protein, 119 aa, Canis lupus familiaris; identical to SEQ ID NO: 27

SEQ ID NO: 44 - protein, 213 aa, Canis lupus familiaris
MAAPAVSGLSRQVRCFSTSVVRPFSKLVRPPVQIYGIEGRYATALYSAASKQNKLEQVEKELLRVAQILKEPKMAASIMNPYIKRSVKVKSLNDMTAKERFSPITSNLINLLAENGRLNNTPGVISAFSTMMSVHRGEVPCTVTTASPLDEATLTELKTVLKSFLSKGQVLKLEVKVDPSIMGGMIVRIGEKYADMSARTKIQKLSRAMREVF

SEQ ID NO: 45 - protein, 518 aa, Canis lupus familiaris
MAAPSRLLIRGGRVVNADLSQAADVLVEDGPMRALGRHLLPPGGAAGLRVLDASGKLVLPGGIDTHTHMQFPFMGSRSVDDFLQGTQAALAGGTTMIIDFAIPQKGGSLIQAFETWRSWADPKVCCDYSLHVAVTWWSDQVKEEMKILTQDKGVNSFKMFMAYKDLYMVRDEELYAAFSQCKEIGAIALVHAENGDLIAEGAKKMLALGITGPEGHELCRPEAVEAEATLRAITIASAVNCPLYVVHVMSKSAAKVIADARRDGKVVYGEPIAASLGTDGTHYWHKEWHHAAHHVMGPPLRPDPSTPDFLMNLLANGDLTTTGTDHCTFNTCQKALGKDDFTKIPNGVNGVEDRMSVIWEKGVHSGKMDENRFVAVTSTNAAKVFNLYPRKGRIAVGSDADIVIWDPKATRTISAKTHHQAVNFNIFEGMVCHGVPVVTISRGKVVYEAGVFNVTAGDGKFIPRKPFAEYIYKRIKQRDQTCTPIPVERKPYKGEVVTVKSRETEEDSAAGMRKQAGP

SEQ ID NO: 46 - protein, 255 aa, Felis catus; identical to SEQ ID NO: 18

SEQ ID NO: 47 - protein, 255 aa, Felis catus
MLQDVLFSSCCSLLVQVAFHDEMVESMKKVAGMDVELTVEERNLLSVAYKNVIGARRASWRIISSIEQKEENKGGEDKLKMIREYRQMVETELKLICCDILDVLDKHLIPAANTGESKVFYYKMKGDYHRYLAEFATGNDRKEAAENSLVAYKAASDIAMTELPPTHPIRLGLALNFSVFYYEILNSPDRACRLAKAAFDDAIAELDTLSEESYKDSTLIMQLLRDNLTLWTSDMQGDGEEQNKEALQDVEDENQ

SEQ ID NO: 48 - protein, 240 aa, Felis catus; identical to SEQ ID NO: 19

SEQ ID NO: 49 - protein, 245 aa, Felis catus; identical to SEQ ID NO: 22

SEQ ID NO: 50 - protein, 245 aa, Felis catus; identical to SEQ ID NO: 36

SEQ ID NO: 51 - protein, 244 aa, Felis catus; identical to SEQ ID NO: 37

SEQ ID NO: 52 - protein, 246 aa, Felis catus; identical to SEQ ID NO: 38

SEQ ID NO: 53 - protein, 247 aa, Felis catus; identical to SEQ ID NO: 25

SEQ ID NO: 54 - protein, 248 aa, Felis catus
MERASLIQKAKLAEQAERYEDMAAFMKSAVEKGEELSCEERNLLSVAYKNVVGGQRAAWRVLSSIEQKGNEESSEEKGPEVREYREKVETELRGVCDTVLGLLDTHLIKEAGDAESRVFYLKMKGDYYRYLAEVATGDDKKRIIDSARSAYQEAMDISKKEMPPTNPIRLGLALNFSVFHYEIANSPEEAISLAKTTFDEAMADLHTLSEDSYKDSTLIMQLLRDNLTLWTADNAGEEGGEAPEEPQS

SEQ ID NO: 55 - protein, 500 aa, Felis catus
MGAGGPRRGAGPPDGGWGWAVLGACFVITGFAYGFPKAVSVFFRALMRDFGAGYSDTAWVSSIMLAMLYGTGPVSSILVTRFGCRPVMLVGGLLASAGMVLASFATRLLELYLTAGVLTGLGLALNFQPSLIMLGLYFERRRPLANGLAAAGSPVFLSALSPLGQQLLEHFGWRGGFLLLGGLLLHCCACGAVMRPPPGPGPRPRGDSAEDAPGEAEADRAGLRLREAPPGGRTRRRLLDVAVCADRAFGVYAITKFLMALGLFVPAILLVNYAKDAGVPDADAAFLLSIVGFVDIVARPACGALAGLARLRPHVAYLFSLALMANGLTDLSSARARSYGALVAFCVAFGLSYGMVGALQFEVLMAAVGSHRFPSALGLVLLVEAVAVLIGPPSAGRLVDALKNYEIIFYLAGSEVALAGIFMAVATKCCLRRSKDTPPSQGAQGGASDTEDAEAQEDAEALPAGAEEPGSLQALEAPSPGAGPGEPKAEAEAGVDPESV

SEQ ID NO: 56 - protein, 460 aa, Felis catus
MGGAVVDEGPTGIKAPDGGWGWAVLFGCFVITGFSYAFPKAVSVFFKELMREFGIGYSDTAWISSILLAMLYGTGPLCSVCVNRFGCRPVMLAGGLLASLGMVAASFCGSIIQLYLTTGVITGLGLALNFQPSLIMLNRYFNKRRPMANGLAAAGSPVFLCALSPLGQLLQDHYGWRGGFLILGGLLLNCCVCAALMRPLEASRPGSGPGPQRPARRLLDLSVFRDRGFVIYAAAASIMVLGLFVPPVFVVSYAKDLGVPDTQAAFLLTVLGFIDIFARPAAGFITGLKKVRPYSVYLFSFSMFFNGFTDLTGSTASDYGGLVVFCIFFGISYGMVGALQFEVLMAIVGTQKFSSAIGLVLLLEAIAVLIGPPSGGKLLDATHVYQYVFLLAGAEVVASSLVLVLGNFFCIKKRPEAAVEEGERHKPPADVRVDSREVEHFLKAEPEKNGEVVHTPETSV

SEQ ID NO: 57 - protein, 480 aa, Felis catus
MGGAVVDEGPTGIKAPDGGWGWAVLFGCFVITGFSYAFPKAVSVFFKELMREFGIGYSDTAWISSILLAMLYGTGPLCSVCVNRFGCRPVMLAGGLLASLGMVAASFCGSIIQLYLTTGVITGEWGPAGSGAGHGTLTPQWPGLGLALNFQPSLIMLNRYFNKRRPMANGLAAAGSPVFLCALSPLGQLLQDHYGWRGGFLILGGLLLNCCVCAALMRPLEASRPGSGPGPQRPARRLLDLSVFRDRGFVIYAAAASIMVLGLFVPPVFVVSYAKDLGVPDTQAAFLLTVLGFIDIFARPAAGFITGLKKVRPYSVYLFSFSMFFNGFTDLTGSTASDYGGLVVFCIFFGISYGMVGALQFEVLMAIVGTQKFSSAIGLVLLLEAIAVLIGPPSGGKLLDATHVYQYVFLLAGAEVVASSLVLVLGNFFCIKKRPEAAVEEGERHKPPADVRVDSREVEHFLKAEPEKNGEVVHTPETSV

SEQ ID NO: 58 - protein, 327 aa, Felis catus
MQEPGSEEEFHSLGFYRMTTRDLTMAMIFFLQTTVGILGNFSVFYYYLFLYLTGYKLRCTDLIVKYLTVANLLVIFSKGIPQTMASFGLPHFLDDFGCKLVFFVHRVGRDVAIGTTCLLTVFQVIMISPGDSRWAQLKIKAPKYMGTSNIFCWVLNIVRSIVVPFHLTDKRNNINVTKKIDQDYCYAISSDKIAQSFYVPLLLSHDGFCLGLMLWASGSMVFILHSHKQRVQYIRRNNLSPRSSPESRATRSILVLAFFFLSLWMLSSIFHMCFSVFNNPSLWLRNTSTILTMCFPTLSPYILMRHDPRVSTLYSAWIRKQNRLNLS

SEQ ID NO: 59 - protein, 241 aa, Felis catus
MFPLLSGAGLVVLNLVTSARSLKTEPFIGSGDQPLFHGADRSDFAVMIPPGGTECFWQFAYQNGYFYFSYEVQRTLGMSHDRHVAATAHTPQGFLIDSSQDVRGQINFSIKETGFYQLCLNNQQNHFGSVQVYLNFGVFYEGPEMDHKQKNERKQLNDTLDAIEESTQKMQNNIFHMWRYYNFARMRKMADFFLLQSNYNYVNWWSTAQSFVIVLSGILQLYFLKRLFNVPKVTDTKKPRC

SEQ ID NO: 60 - protein, 239 aa, Felis catus
MFPLLSGAGLVVLNLVTSARSLKTEPFIGSGDQPLFHGADRSDFAVMIPPGGTECFWQFAYQNGYFYFSYERTLGMSHDRHVAATAHTPQGFLIDSSQDVRGQINFSIKETGFYQLCLNNQQNHFGSVQVYLNFGVFYEGPEMDHKQKNERKQLNDTLDAIEESTQKMQNNIFHMWRYYNFARMRKMADFFLLQSNYNYVNWWSTAQSFVIVLSGILQLYFLKRLFNVPKVTDTKKPRC

SEQ ID NO: 61 - protein, 119 aa, Felis catus; identical to SEQ ID NO: 27

SEQ ID NO: 62 - protein, 112 aa, Felis catus
MKLSHETVTIELKNGTQVHGTITGVDVSMNTHLKAVKMTLKNREPVQLETLSIRGNNIRYFILPDSLPLDTLLVDVEPKVKSKKREAVAGRGRGRGRGRGRGRGRGRGGPRR

SEQ ID NO: 63 - protein, 213 aa, Felis catus
MASSAVSGLSRQVRCFSTSVVRPFAKLVRPPVQIYGIEGRYATALYSAASKQNKLEQVEKELLRVAQILKEPKMAASIMNPYVKRSVKVKSLNDMTAKERFSPLTCNLINLLAENGRLNNTPGVVSAFSTMMSVHRGEVPCTVTTASPLDEPTLAELRTVLKSFLSKGQVLKLEVKIDPSIMGGMIVRIGEKYADMSAKTKIQKLSRAMREIF

SEQ ID NO: 64 - protein, 519 aa, Felis catus
MAAPSRLLIRGGRVVNDDLSQVADVLVEDGVVRALGRDLLPPGGAPAGLRVLDAAGKLVLPGGIDTHTHMQFPFMGARSVDDFHQGTKAALAGGTTMIIDFAIPQKGGSLIKAFETWRSWADPKVCCDYSLHVAVTWWSDQVKEEMKILTQDKGVNSFKMFMAYKDLYMVRDEELYAAFSQCKEIGAIAQVHAENGDLIAEGAKKMLALGITGPEGHELCRPEAVEAEATLRAITIASAVNCPLYIVHVMSKSAAKVIADARRDGKVVYGEPIAASLGTDGTHYWHKDWHHAAHHVMGPPLRPDPSTPDFLMNLLANGDLTTTGTDHCTFNTCQKALGKDDFTKIPNGVNGVEDRMSVIWEKGVHSGKMDENRFVAVTSTNAAKVFNLYPRKGRIAVGSDADIVIWDPKATRTISARTHHQAVNFNIFEGMVCHGVPLVTISRGKVVYEAGVLSVTAGDGKFIPRKPFAEYIYKRIKQRDQTCTPTPVEREPYKGEVVTLKTRETKEDAAAGTRKQAHP

SEQ ID NO: 65 - protein, 513 aa, Felis catus
MAAPSRLLIRGGRVVNDDLSQVADVLVEDGVVRALGRDLLPPGGAPAGLRVLDAAGKLVLPGGIDTHTHMQFPFMGARSVDDFHQGTKAALAGGTTMIIDFAIPQKGGSLIKAFETWRSWADPKVCCDYSLHVAVTWWSDQVKEEMKILTQDKGVNSFKMFMAYKDLYMVRDEELYAAFSQCKEIGAIAQVHAENGDLIAEGAKKMLALGITGPEGHELCRPEAVEAEATLRAITIASAVNCPLYIVHVMSKSAAKVIADARRDGKVVYGEPIAASLGTDGTHYWHKDWHHAAHHVMGPPLRPDPSTPDFLMNLLANGDLTTTGTDHCTFNTCQKALGKDDFTKIPNGVNGVEDRMSVIWEKGVHSGKMDENRFVAVTSTNAAKVFNLYPRKGRIAVGSDADIVIWDPKATRTISARTHHQAVNFNIFEGMVCHGVPLVTISRGKVVYEAGVLSVTAGDGKFIPRKPFAEYIYKRIKQRDQVKSEKRILLFPSLLSVVSPWRNRPHFNSPRCF

SEQ ID NO: 66 - protein, 466 aa, Mus musculus
MGAGALALGASEPCNLSSAAPLPDGAATAARLLVLASPPASLLPPASEGSAPLSQQWTAGMGLLLALIVLLIVVGNVLVIVAIAKTPRLQTLTNLFIMSLASADLVMGLLVVPFGATIVVWGRWEYGSFFCELWTSVDVLCVTASIETLCVIALDRYLAITSPFRYQSLLTRARARALVCTVWAISALVSFLPILMHWWRAESDEARRCYNDPKCCDFVTNRAYAIASSVVSFYVPLCIMAFVYLRVFREAQKQVKKIDSCERRFLGGPARPPSPEPSPSPGPPRPADSLANGRSSKRRPSRLVALREQKALKTLGIIMGVFTLCWLPFFLANVVKAFHRDLVPDRLFVFFNWLGYANSAFNPIIYCRSPDFRKAFQRLLCCARRAACRRRAAHGDRPRASGCLARAGPPPSPGAPSDDDDDDAGTTPPARLLEPWTGCNGGTTTVDSDSSLDEPGRQGFSSESKV

SEQ ID NO: 67 - protein, 477 aa, Homo sapiens
MGAGVLVLGASEPGNLSSAAPLPDGAATAARLLVPASPPASLLPPASESPEPLSQQWTAGMGLLMALIVLLIVAGNVLVIVAIAKTPRLQTLTNLFIMSLASADLVMGLLVVPFGATIVVWGRWEYGSFFCELWTSVDVLCVTASIETLCVIALDRYLAITSPFRYQSLLTRARARGLVCTVWAISALVSFLPILMHWWRAESDEARRCYNDPKCCDFVTNRAYAIASSVVSFYVPLCIMAFVYLRVFREAQKQVKKIDSCERRFLGGPARPPSPSPSPVPAPAPPPGPPRPAAAAATAPLANGRAGKRRPSRLVALREQKALKTLGIIMGVFTLCWLPFFLANVVKAFHRELVPDRLFVFFNWLGYANSAFNPIIYCRSPDFRKAFQRLLCCARRAARRRHATHGDRPRASGCLARPGPPPSPGAASDDDDDDVVGATPPARLLEPWAGCNGGAAADSDSSLDEPCRPGFASESKV

SEQ ID NO: 68 - protein, 473 aa, Canis lupus familiaris
MGAGALALGASEPCNLSSAAPLPDGAATAARLLVPASPSASPLAPTSEGPAPLSQQWTAGIGLLMALIVLLIVAGNVLVIAAIAKTPRLQTLTNLFIMSLASADLVMGLLVVPFGATIVMRGRWEYGSFLCELWTSVDVLCVTASIETLCVIALDRYLAITAPFRYQSLLTRARARALVCTVWAISALVSFLPILMHWWRAGGDEARRCYNDPKCCDFVTNRAYAIASSVVSFYVPLCIMAFVYLRVFREAQKQVKKIDSCERRFLGGPARPPAPPPAPAPAPPPAPGSPRPAAAAPLANGRVGRRRPSRLVALREQKALKTLGIIMGVFTLCWLPFFLANVVKAFHRDLVPDRLFVFFNWLGYANSAFNPIIYCRSPDFRRAFQRLLCCARRAARGSHGAAGDPPRARPPPSPGAASDDDDDDEDDAGAGAGAAPPARLLEPWAGCNGGAAADSDSSLDGAGSPAGASESRV

SEQ ID NO: 69 - protein, 474 aa, Felis catus
MGAGALALGASEPCNLSSAAPLPDGAATAARLLVPASPSASPLTPTSEGPAPLSQQWTAGIGLLMALIVLLIVAGNVLVIVAIAKTPRLQTLTNLFIMSLASADLVMGLLVVPFGATIVMRGRWEYGSFFCELWTSVDVLCVTASIETLCVIALDRYLAITSPFRYQSLLTRARARALVCTVWAISALVSFLPILMHWWRAEGDEARRCYNDPKCCDFVTNRAYAIASSVVSFYVPLCIMAFVYLRVFREAQKQVKKIDSCERRFLSGPARPPSPAPAPGSPRPAATAAAAAAAAPLANGRISKRRPSRLVALREQKALKTLGIIMGVFTLCWLPFFLANVVKAFHRDLVPDRLFVFFNWLGYANSAFNPIIYCRSPDFRKAFQRLLCFARRAARGGHAAAGDRPRASGCLPGTRPPPSPGAASDEDDDDDVGAAPPARLLEPWAGCNGGAAAADSDSSLDEPGRPAGASESKV

SEQ ID NO: 70 - protein, 255 aa, Mus musculus; identical to SEQ ID NO: 18

SEQ ID NO: 71 - protein, 246 aa, Mus musculus
MTMDKSELVQKAKLAEQAERYDDMAAAMKAVTEQGHELSNEERNLLSVAYKNVVGARRSSWRVISSIEQKTERNEKKQQMGKEYREKIEAELQDICNDVLELLDKYLILNATQAESKVFYLKMKGDYFRYLSEVASGENKQTTVSNSQQAYQEAFEISKKEMQPTHPIRLGLALNFSVFYYEILNSPEKACSLAKTAFDEAIAELDTLNEESYKDSTLIMQLLRDNLTLWTSENQGDEGDAGEGEN

SEQ ID NO: 72 - protein, 245 aa, Mus musculus
MDKNELVQKAKLAEQAERYDDMAACMKSVTEQGAELSNEERNLLSVAYKNVVGARRSSWRVVSSIEQKTEGAEKKQQMAREYREKIETELRDICNDVLSLLEKFLIPNASQPESKVFYLKMKGDYYRYLAEVAAGDDKKGIVDQSQQAYQEAFEISKKEMQPTHPIRLGLALNFSVFYYEILNSPEKACSLAKTAFDEAIAELDTLSEESYKDSTLIMQLLRDNLTLWTSDTQGDEAEAGEGGEN

SEQ ID NO: 73 - protein, 245 aa, Mus musculus
MEKTELIQKAKLAEQAERYDDMATCMKAVTEQGAELSNEERNLLSVAYKNVVGGRRSAWRVISSIEQKTDTSDKKLQLIKDYREKVESELRSICTTVLELLDKYLIANATNPESKVFYLKMKGDYFRYLAEVACGDDRKQTIENSQGAYQEAFDISKKEMQPTHPIRLGLALNFSVFYYEILNNPELACTLAKTAFDEAIAELDTLNEDSYKDSTLIMQLLRDNLTLWTSDSAGEECDAAEGAEN

SEQ ID NO: 74 - protein, 246 aa, Mus musculus; identical to SEQ ID NO: 38

SEQ ID NO: 75 - protein, 247 aa, Mus musculus; identical to SEQ ID NO: 25

SEQ ID NO: 76 - protein, 248 aa, Mus musculus
MERASLIQKAKLAEQAERYEDMAAFMKSAVEKGEELSCEERNLLSVAYKNVVGGQRAAWRVLSSIEQKSNEEGSEEKGPEVKEYREKVETELRGVCDTVLGLLDSHLIKGAGDAESRVFYLKMKGDYYRYLAEVATGDDKKRIIDSARSAYQEAMDISKKEMPPTNPIRLGLALNFSVFHYEIANSPEEAISLAKTTFDEAMADLHTLSEDSYKDSTLIMQLLRDNLTLWTADSAGEEGGEAPEEPQS

SEQ ID NO: 77 - protein, 492 aa, Mus musculus
MGAGGPRRGAGPPDGGWGWVVLGACFVVTGFAYGFPKAVSVFFRELKRDFGAGYSDTAWVSSIMLAMLYGTGPLSSILVTRFGCRPVMLAGGLLASAGMILASFASRLVELYLTAGVLTGLGLALNFQPSLIMLGLYFERRRPLANGLAAAGSPVFLSMLSPLGQLLGERFGWRGGFLLFGGLLLHCCACGAVMRPPPGPPPRRDPSPHGGPARRRRLLDVAVCTDRAFVVYVVTKFLMALGLFVPAILLVNYAKDAGVPDAEAAFLLSIVGFVDIVARPACGALAGLGRLRPHVPYLFSLALLANGLTDLISARARSYGTLVAFCIAFGLSYGMVGALQFEVLMATVGAPRFPSALGLVLLVEAVAVLIGPPSAGRLVDALKNYEIIFYLAGSEVALAGVFMAVTTYCCLRCSKNISSGRSAEGGASDPEDVEAERDSEPMPASTEEPGSLEALEVLSPRAGSPEQEPEEEAVPELDHESIGGHEARGQKA

SEQ ID NO: 78 - protein, 470 aa, Mus musculus
MGGAVVDEGPTGIKAPDGGWGWAVLFGCFIITGFSYAFPKAVSVFFKELMHEFGIGYSDTAWISSILLAMLYGTGPLCSVCVNRFGCRPVMLVGGLFASLGMVAASFCRSIIQIYLTTGVITGLGLALNFQPSLIMLNRYFNKRRPIANGLAAAGSPVFLCALSPLGQLLQDHYGWRGGFLILGGLLLNCCVCAALMRPLVAPQVGGGTEPRGPQRPPQRLLDLSVFRDRGFLIYAVAASIMVLGLFVPPVFVVSYAKDMGVPDTKAAFLLTILGFIDIFARPTAGFITGLKKVRPYSVYLFSFAMFFNGFTDLTGSTATDYGGLVVFCIFFGISYGMVGALQFEVLMAIVGTQKFSSAIGLVLLLEAVAVLIGPPSGGKLLDATKVYKYVFILAGAEVLTSSLVLLLGNFFCIGKRKRPEVTEPEEVASEEKLHKPPVDVGVDSREVEHFLKAEPEKNGEVVHTPETSV

SEQ ID NO: 79 - protein, 119 aa, Mus musculus; identical to SEQ ID NO: 27

SEQ ID NO: 80 - protein, 213 aa, Mus musculus
MAAPAASGLSRQVRSFSTSVVRPFAKLVRPPVQVYGIEGRYATALYSAASKEKKLDQVEKELLRVGQLLKDPKVSLAVLNPYIKRTVKVKSLNDITKREKFSPLTANLMNLLAENGRLGNTQGIISAFSTIMSVHRGEVPCTVTTASPLDDAVLSELKTVLKSFLSPNQILKLEIKTDPSIMGGMIVRIGEKYVDMSAKSKIQKLSKAMREML